European Patent Application EP 4 428 143 A1, published September 11, 2024. Title: Peptide Having Physiological Activity and Use Thereof. Applicant: CAREGEN CO., LTD. The sequence listing filed with the application follows.

SEQUENCE LISTING (23 sequences)

SEQ ID NO: 1 - protein, 11 aa, synthetic construct
  REGION 1..11: note = peptide having cartilage regeneration activity
NAISVLYFDDS

SEQ ID NO: 2 - DNA, 23 bp, synthetic construct
  misc_feature 1..23: note = forward primer for hCOL2A1 gene
  source 1..23: mol_type = other DNA
ctatctggacgaagcagctggca

SEQ ID NO: 3 - DNA, 22 bp, synthetic construct
  misc_feature 1..22: note = reverse primer for hCOL2A1 gene
  source 1..22: mol_type = other DNA
atgggtgcaatgtcaatgatgg

SEQ ID NO: 4 - DNA, 20 bp, synthetic construct
  misc_feature 1..20: note = forward primer for hCOMP gene
  source 1..20: mol_type = other DNA
aactcagggcaggaggatgt

SEQ ID NO: 5 - DNA, 20 bp, synthetic construct
  misc_feature 1..20: note = reverse primer for hCOMP gene
  source 1..20: mol_type = other DNA
tgtccttttggtcgtcgttc

SEQ ID NO: 6 - DNA, 20 bp, synthetic construct
  misc_feature 1..20: note = forward primer for hPCP gene
  source 1..20: mol_type = other DNA
tgagtcctcaagcctcctgt

SEQ ID NO: 7 - DNA, 20 bp, synthetic construct
  misc_feature 1..20: note = reverse primer for hPCP gene
  source 1..20: mol_type = other DNA
gtgccagatcatcaccacac

SEQ ID NO: 8 - DNA, 20 bp, synthetic construct
  misc_feature 1..20: note = forward primer for GAPDH gene
  source 1..20: mol_type = other DNA
accacagtccatgccatcac

SEQ ID NO: 9 - DNA, 20 bp, synthetic construct
  misc_feature 1..20: note = reverse primer for GAPDH gene
  source 1..20: mol_type = other DNA
tccaccaccctgttgctgta

SEQ ID NO: 10 - DNA, 20 bp, synthetic construct
  misc_feature 1..20: note = forward primer for hSox9 gene
  source 1..20: mol_type = other DNA
gcggaggaagtcggtgaaga

SEQ ID NO: 11 - DNA, 20 bp, synthetic construct
  misc_feature 1..20: note = reverse primer for hSox9 gene
  source 1..20: mol_type = other DNA
ccctctcgcttcaggtcagc

SEQ ID NO: 12 - DNA, 20 bp, synthetic construct
  misc_feature 1..20: note = forward primer for hCOL11A gene
  source 1..20: mol_type = other DNA
ccagcccgaacttgtaaaga

SEQ ID NO: 13 - DNA, 20 bp, synthetic construct
  misc_feature 1..20: note = reverse primer for hCOL11A gene
  source 1..20: mol_type = other DNA
tggacgcacaaccatcatac

SEQ ID NO: 14 - DNA, 20 bp, synthetic construct
  misc_feature 1..20: note = forward primer for hACP gene
  source 1..20: mol_type = other DNA
cactgttaccgccacttccc

SEQ ID NO: 15 - DNA, 20 bp, synthetic construct
  misc_feature 1..20: note = reverse primer for hACP gene
  source 1..20: mol_type = other DNA
accagcggaagtccccttcg

SEQ ID NO: 16 - DNA, 20 bp, synthetic construct
  misc_feature 1..20: note = forward primer for hACAN gene
  source 1..20: mol_type = other DNA
gcaggctatgagcagtgtga

SEQ ID NO: 17 - DNA, 20 bp, synthetic construct
  misc_feature 1..20: note = reverse primer for hACAN gene
  source 1..20: mol_type = other DNA
gcatacctcggaagcagaag

SEQ ID NO: 18 - DNA, 20 bp, synthetic construct
  misc_feature 1..20: note = forward primer for TNF-alpha gene
  source 1..20: mol_type = other DNA
cgtcagccgatttgctatct

SEQ ID NO: 19 - DNA, 20 bp, synthetic construct
  misc_feature 1..20: note = reverse primer for TNF-alpha gene
  source 1..20: mol_type = other DNA
cggactccgcaaagtctaag

SEQ ID NO: 20 - DNA, 20 bp, synthetic construct
  misc_feature 1..20: note = forward primer for IL-1beta gene
  source 1..20: mol_type = other DNA
caaggagaaccaagcaacga

SEQ ID NO: 21 - DNA, 20 bp, synthetic construct
  misc_feature 1..20: note = reverse primer for IL-1beta gene
  source 1..20: mol_type = other DNA
ttggccgaggactaaggagt

SEQ ID NO: 22 - DNA, 20 bp, synthetic construct
  misc_feature 1..20: note = forward primer for Cox2 gene
  source 1..20: mol_type = other DNA
tgagtggtagccagcaaagc

SEQ ID NO: 23 - DNA, 20 bp, synthetic construct
  misc_feature 1..20: note = reverse primer for Cox2 gene
  source 1..20: mol_type = other DNA
ctgcagtccaggttcaatgg